European Patent Application EP 4 140 502 A1, published March 1, 2023. Title: 溶瘤病毒与免疫检查点抑制剂联合治疗肿瘤. Applicant: 上海荣瑞医药科技有限公司. The sequence listing filed with the application follows.

SEQUENCE LISTING (13 sequences)

SEQ ID NO: 1 - DNA, 690 bp, 水疱性口炎病毒印第安纳株(VSV MuddSummer)
atgagttccttaaagaagattctcggtctgaaggggaaaggtaagaaatctaagaaattagggatcgcaccacccccttatgaagaggacactagcatggagtatgctccgagcgctccaattgacaaatcctattttggagttgacgagatggacacctatgatccgaatcaattaagatatgagaaattcttctttacagtgaaaatgacggttagatctaatcgtccgttcagaacatactcagatgtggcagccgctgtatcccattgggatcacatgtacatcggaatggcagggaaacgtcccttctacaaaatcttggcttttttgggttcttctaatctaaaggccactccagcggtattggcagatcaaggtcaaccagagtatcacgctcactgcgaaggcagggcttatttgccacataggatggggaagacccctcccatgctcaatgtaccagagcacttcagaagaccattcaatataggtctttacaagggaacgattgagctcacaatgaccatctacgatgatgagtcactggaagcagctcctatgatctgggatcatttcaattcttccaaattttctgatttcagagagaaggccttaatgtttggcctgattgtcgagaaaaaggcatctggagcgtgggtcctggactctatcggccacttcaaatga

SEQ ID NO: 2 - protein, 229 aa, 水疱性口炎病毒印第安纳株(VSV MuddSummer)
MSSLKKILGLKGKGKKSKKLGIAPPPYEEDTSMEYAPSAPIDKSYFGVDEMDTYDPNQLRYEKFFFTVKMTVRSNRPFRTYSDVAAAVSHWDHMYIGMAGKRPFYKILAFLGSSNLKATPAVLADQGQPEYHAHCEGRAYLPHRMGKTPPMLNVPEHFRRPFNIGLYKGTIELTMTIYDDESLEAAPMIWDHFNSSKFSDFREKALMFGLIVEKKASGAWVLDSISHFK

SEQ ID NO: 3 - DNA, 687 bp, 人工序列（Artificial Sequence）
  基质蛋白M（M51R，ΔL111，V221F，S226R）
atgagttccttaaagaagattctcggtctgaaggggaaaggtaagaaatctaagaaattagggatcgcaccacccccttatgaagaggacactagcatggagtatgctccgagcgctccaattgacaaatcctattttggagttgacgagatggacacctatgatccgaatcaattaagatatgagaaattcttctttacagtgaaaatgacggttagatctaatcgtccgttcagaacatactcagatgtggcagccgctgtatcccattgggatcacatgtacatcggaatggcagggaaacgtcccttctacaaaatcttggctttgggttcttctaatctaaaggccactccagcggtattggcagatcaaggtcaaccagagtatcacgctcactgcgaaggcagggcttatttgccacataggatggggaagacccctcccatgctcaatgtaccagagcacttcagaagaccattcaatataggtctttacaagggaacgattgagctcacaatgaccatctacgatgatgagtcactggaagcagctcctatgatctgggatcatttcaattcttccaaattttctgatttcagagagaaggccttaatgtttggcctgattgtcgagaaaaaggcatctggagcgtgggtcctggactctatcggccacttcaaatga

SEQ ID NO: 4 - protein, 228 aa, 人工序列（Artificial Sequence）
  基质蛋白M（M51R，ΔL111，V221F，S226R）（PRT）
MSSLKKILGLKGKGKKSKKLGIAPPPYEEDTSMEYAPSAPIDKSYFGVDERDTYDPNQLRYEKFFFTVKMTVRSNRPFRTYSDVAAAVSHWDHMYIGMAGKRPFYKILAFGSSNLKATPAVLADQGQPEYHAHCEGRAYLPHRMGKTPPMLNVPEHFRRPFNIGLYKGTIELTMTIYDDESLEAAPMIWDHFNSSKFSDFREKALMFGLIVEKKASGAWFLDSIRHFK

SEQ ID NO: 5 - DNA, 20 bp, 人工序列（Artificial Sequence）
  引物1
aaaaaagtaacagatatcac

SEQ ID NO: 6 - DNA, 24 bp, 人工序列（Artificial Sequence）
  引物2
acatttttccagtttcctttttgg

SEQ ID NO: 7 - protein, 228 aa, 人工序列（Artificial Sequence）
  基质蛋白M（ΔL111）
MSSLKKILGLKGKGKKSKKLGIAPPPYEEDTSMEYAPSAPIDKSYFGVDEMDTYDPNQLRYEKFFFTVKMTVRSNRPFRTYSDVAAAVSHWDHMYIGMAGKRPFYKILAFGSSNLKATPAVLADQGQPEYHAHCEGRAYLPHRMGKTPPMLNVPEHFRRPFNIGLYKGTIELTMTIYDDESLEAAPMIWDHFNSSKFSDFREKALMFGLIVEKKASGAWVLDSISHFK

SEQ ID NO: 8 - protein, 228 aa, 人工序列（Artificial Sequence）
  基质蛋白M（ΔL111，M51R）
MSSLKKILGLKGKGKKSKKLGIAPPPYEEDTSMEYAPSAPIDKSYFGVDERDTYDPNQLRYEKFFFTVKMTVRSNRPFRTYSDVAAAVSHWDHMYIGMAGKRPFYKILAFGSSNLKATPAVLADQGQPEYHAHCEGRAYLPHRMGKTPPMLNVPEHFRRPFNIGLYKGTIELTMTIYDDESLEAAPMIWDHFNSSKFSDFREKALMFGLIVEKKASGAWVLDSISHFK

SEQ ID NO: 9 - protein, 228 aa, 人工序列（Artificial Sequence）
  基质蛋白M（ΔL111，V221F）
MSSLKKILGLKGKGKKSKKLGIAPPPYEEDTSMEYAPSAPIDKSYFGVDEMDTYDPNQLRYEKFFFTVKMTVRSNRPFRTYSDVAAAVSHWDHMYIGMAGKRPFYKILAFGSSNLKATPAVLADQGQPEYHAHCEGRAYLPHRMGKTPPMLNVPEHFRRPFNIGLYKGTIELTMTIYDDESLEAAPMIWDHFNSSKFSDFREKALMFGLIVEKKASGAWFLDSISHFK

SEQ ID NO: 10 - protein, 228 aa, 人工序列（Artificial Sequence）
  基质蛋白M（ΔL111，S226R）
MSSLKKILGLKGKGKKSKKLGIAPPPYEEDTSMEYAPSAPIDKSYFGVDEMDTYDPNQLRYEKFFFTVKMTVRSNRPFRTYSDVAAAVSHWDHMYIGMAGKRPFYKILAFGSSNLKATPAVLADQGQPEYHAHCEGRAYLPHRMGKTPPMLNVPEHFRRPFNIGLYKGTIELTMTIYDDESLEAAPMIWDHFNSSKFSDFREKALMFGLIVEKKASGAWVLDSIRHFK

SEQ ID NO: 11 - protein, 228 aa, 人工序列（Artificial Sequence）
  基质蛋白M（ΔL111，V221F，S226R）
MSSLKKILGLKGKGKKSKKLGIAPPPYEEDTSMEYAPSAPIDKSYFGVDEMDTYDPNQLRYEKFFFTVKMTVRSNRPFRTYSDVAAAVSHWDHMYIGMAGKRPFYKILAFGSSNLKATPAVLADQGQPEYHAHCEGRAYLPHRMGKTPPMLNVPEHFRRPFNIGLYKGTIELTMTIYDDESLEAAPMIWDHFNSSKFSDFREKALMFGLIVEKKASGAWFLDSIRHFK

SEQ ID NO: 12 - protein, 120 aa, 人工序列（Artificial Sequence） [sequence omitted]

SEQ ID NO: 13 - protein, 112 aa, 人工序列（Artificial Sequence）
  PD-1抗体VL
EIVLTQSPATLSLSPGERATLSCRASKGVSTSGYSYLHWYQQKPGQAPRLLIYLASYLESGVPARFSGSGSGTDFTLTISSLEPEDFAVYYCQHSRDLPLTFGGGTKVEIKR